European Patent Application EP 4 495 244 A1, published January 22, 2025. Title: 改変型プロテイングルタミナーゼ. Applicant: Amano Enzyme Inc. Application JP. The sequence listing filed with the application follows.

SEQUENCE LISTING (26 sequences)

SEQ ID NO: 1 - protein, 185 aa, Chryseobacterium proteolyticum
LASVIPDVATLNSLFNQIKNQSCGTSTASSPCITFRYPVDGCYARAHKMRQILMNNGYDCEKQFVYGNLKASTGTCCVAWSYHVAILVSYKNASGVTEKRIIDPSLFSSGPVTDTAWRNACVNTSCGSASVSSYANTAGNVYYRSPSNSYLYDNNLINTNCVLTKFSLLSGCSPSPAPDVSSCGF

SEQ ID NO: 2 - protein, 320 aa, Chryseobacterium proteolyticum
MKNLFLSMMAFVTVLTFNSCADSNGNQEINGKEKLSVNDSKLKDFGKTVPVGIDEENGMIKVSFMLTAQFYEIKPTKENEQYIGMLRQAVKNESPVHIFLKPNSNEIGKVESASPEDVRYFKTILTKEVKGQTNKLASVIPDVATLNSLFNQIKNQSCGTSTASSPCITFRYPVDGCYARAHKMRQILMNNGYDCEKQFVYGNLKASTGTCCVAWSYHVAILVSYKNASGVTEKRIIDPSLFSSGPVTDTAWRNACVNTSCGSASVSSYANTAGNVYYRSPSNSYLYDNNLINTNCVLTKFSLLSGCSPSPAPDVSSCGF

SEQ ID NO: 3 - protein, 185 aa, synthetic construct
  REGION 1..185: note = C121V mutation of proteinglutaminase derived from Chryseobacteriumproteolyticum
LASVIPDVATLNSLFNQIKNQSCGTSTASSPCITFRYPVDGCYARAHKMRQILMNNGYDCEKQFVYGNLKASTGTCCVAWSYHVAILVSYKNASGVTEKRIIDPSLFSSGPVTDTAWRNAVVNTSCGSASVSSYANTAGNVYYRSPSNSYLYDNNLINTNCVLTKFSLLSGCSPSPAPDVSSCGF

SEQ ID NO: 4 - protein, 185 aa, synthetic construct
  REGION 1..185: note = C121A mutation of proteinglutaminase derived from Chryseobacteriumproteolyticum
LASVIPDVATLNSLFNQIKNQSCGTSTASSPCITFRYPVDGCYARAHKMRQILMNNGYDCEKQFVYGNLKASTGTCCVAWSYHVAILVSYKNASGVTEKRIIDPSLFSSGPVTDTAWRNAAVNTSCGSASVSSYANTAGNVYYRSPSNSYLYDNNLINTNCVLTKFSLLSGCSPSPAPDVSSCGF

SEQ ID NO: 5 - protein, 185 aa, synthetic construct
  REGION 1..185: note = Y142C mutation of proteinglutaminase derived from Chryseobacteriumproteolyticum
LASVIPDVATLNSLFNQIKNQSCGTSTASSPCITFRYPVDGCYARAHKMRQILMNNGYDCEKQFVYGNLKASTGTCCVAWSYHVAILVSYKNASGVTEKRIIDPSLFSSGPVTDTAWRNACVNTSCGSASVSSYANTAGNVCYRSPSNSYLYDNNLINTNCVLTKFSLLSGCSPSPAPDVSSCGF

SEQ ID NO: 6 - protein, 185 aa, synthetic construct
  REGION 1..185: note = Y142D mutation of proteinglutaminase derived from Chryseobacteriumproteolyticum
LASVIPDVATLNSLFNQIKNQSCGTSTASSPCITFRYPVDGCYARAHKMRQILMNNGYDCEKQFVYGNLKASTGTCCVAWSYHVAILVSYKNASGVTEKRIIDPSLFSSGPVTDTAWRNACVNTSCGSASVSSYANTAGNVDYRSPSNSYLYDNNLINTNCVLTKFSLLSGCSPSPAPDVSSCGF

SEQ ID NO: 7 - protein, 185 aa, Chryseobacterium sp.
AVSVIPNLATLNSLFTQIKNQACGTSTASSPCITFRYPVDGCYARAHKMRQILLNAGYDCEKQFVYGNLRASTGTCCVSWVYHVAILVSFKNASGIVEKRIIDPSLFSSGPVTDAAWRAACTNTSCGSASVSSYANTAGNVYYRSPSGSLLYDNNYVNTNCVLNIFSSLSGCSPSPAPSVASCGF

SEQ ID NO: 8 - protein, 185 aa, Chryseobacterium sp.
AVSVIPNLATLNSLFTQIKNQACGTSTASSPCITFRYPVDGCYARAHKMRQILLNAGYDCEKQFVYGNLRASTGTCCVSWVYHVAILVSFKNASGIVEKRIIDPSLFSSGPVTDTAWRAACTNTSCGSASVSSYANTAGNVYYRSPSGSLLYDNNYVNTNCVLNIFSSLSGCSPSPAPSVASCGF

SEQ ID NO: 9 - protein, 319 aa, Chryseobacterium sp.
MKKFLLSMMVFVTMLSFNACSDSAANQDPNLVAKESNEIAMKDFGKTVPVGIEKEEGKFKVSFMVSAQPYHIKDSKENAGYISMIRQAVENETPVHIFLKTNTTEIAKVDKPTDDDIRYFKSVFNKEERGDSKKAVSVIPNLATLNSLFTQIKNQACGTSTASSPCITFRYPVDGCYARAHKMRQILLNAGYDCEKQFVYGNLRASTGTCCVSWVYHVAILVSFKNASGIVEKRIIDPSLFSSGPVTDAAWRAACTNTSCGSASVSSYANTAGNVYYRSPSGSLLYDNNYVNTNCVLNIFSSLSGCSPSPAPSVASCGF

SEQ ID NO: 10 - protein, 319 aa, Chryseobacterium sp.
MKKFLLSMMVFVTVLSFNSCSDSSANQDPNLVAKESNEIAMKDFGKTVPVGIEKEDGKFKVSFIVSAQPYQIKDTKENAGYISMIKEAVENETPVQVFLKANSNEIAKVDKATADDIRYFKSVFNKEERGDSRKAVSVIPNLATLNSLFTQIKNQACGTSTASSPCITFRYPVDGCYARAHKMRQILLNAGYDCEKQFVYGNLRASTGTCCVSWVYHVAILVSFKNASGIVEKRIIDPSLFSSGPVTDTAWRAACTNTSCGSASVSSYANTAGNVYYRSPSGSLLYDNNYVNTNCVLNIFSSLSGCSPSPAPSVASCGF

SEQ ID NO: 11 - DNA, 558 bp, Chryseobacterium proteolyticum
  source 1..558: mol_type = other DNA
ttggcgagtgtaattcctgatgtagctacattaaattctttattcaatcaaataaagaatcagtcttgcggtacctctacggcgtcctcaccatgcatcacattcagatatcctgtagacggatgttatgcaagagcccataagatgagacaaatcttaatgaacaacggctatgactgtgaaaaacaatttgtatacggaaacctaaaggcatcaacaggaacttgctgtgtggcgtggagctaccacgttgcaatattggtaagctataaaaatgcttccggagtaacggaaaaaagaattattgatccttcactattttcaagcggtcctgtaacagatacagcatggagaaacgcttgcgttaacacctcttgcggatctgcatccgtttcctcttatgctaatactgcaggaaatgtttattacagaagtcctagtaattcttacctgtatgacaacaatctgatcaataccaactgtgtactgactaaattttcactgctttccggatgttctccttcacctgcaccggatgtatccagctgtggattttaa

SEQ ID NO: 12 - DNA, 558 bp, synthetic construct
  misc_feature 1..558: note = DNA coding C121V mutation of proteinglutaminase derived fromChryseobacterium proteolyticum
  source 1..558: mol_type = other DNA
ttggcgagtgtaattcctgatgtagctacattaaattctttattcaatcaaataaagaatcagtcttgcggtacctctacggcgtcctcaccatgcatcacattcagatatcctgtagacggatgttatgcaagagcccataagatgagacaaatcttaatgaacaacggctatgactgtgaaaaacaatttgtatacggaaacctaaaggcatcaacaggaacttgctgtgtggcgtggagctaccacgttgcaatattggtaagctataaaaatgcttccggagtaacggaaaaaagaattattgatccttcactattttcaagcggtcctgtaacagatacagcatggagaaacgctgttgttaacacctcttgcggatctgcatccgtttcctcttatgctaatactgcaggaaatgtttattacagaagtcctagtaattcttacctgtatgacaacaatctgatcaataccaactgtgtactgactaaattttcactgctttccggatgttctccttcacctgcaccggatgtatccagctgtggattttaa

SEQ ID NO: 13 - DNA, 558 bp, synthetic construct
  misc_feature 1..558: note = DNA coding C121A mutation of proteinglutaminase derived fromChryseobacterium proteolyticum
  source 1..558: mol_type = other DNA
ttggcgagtgtaattcctgatgtagctacattaaattctttattcaatcaaataaagaatcagtcttgcggtacctctacggcgtcctcaccatgcatcacattcagatatcctgtagacggatgttatgcaagagcccataagatgagacaaatcttaatgaacaacggctatgactgtgaaaaacaatttgtatacggaaacctaaaggcatcaacaggaacttgctgtgtggcgtggagctaccacgttgcaatattggtaagctataaaaatgcttccggagtaacggaaaaaagaattattgatccttcactattttcaagcggtcctgtaacagatacagcatggagaaacgctgcggttaacacctcttgcggatctgcatccgtttcctcttatgctaatactgcaggaaatgtttattacagaagtcctagtaattcttacctgtatgacaacaatctgatcaataccaactgtgtactgactaaattttcactgctttccggatgttctccttcacctgcaccggatgtatccagctgtggattttaa

SEQ ID NO: 14 - DNA, 558 bp, synthetic construct
  misc_feature 1..558: note = DNA coding Y142C mutation of proteinglutaminase derived fromChryseobacterium proteolyticum
  source 1..558: mol_type = other DNA
ttggcgagtgtaattcctgatgtagctacattaaattctttattcaatcaaataaagaatcagtcttgcggtacctctacggcgtcctcaccatgcatcacattcagatatcctgtagacggatgttatgcaagagcccataagatgagacaaatcttaatgaacaacggctatgactgtgaaaaacaatttgtatacggaaacctaaaggcatcaacaggaacttgctgtgtggcgtggagctaccacgttgcaatattggtaagctataaaaatgcttccggagtaacggaaaaaagaattattgatccttcactattttcaagcggtcctgtaacagatacagcatggagaaacgcttgcgttaacacctcttgcggatctgcatccgtttcctcttatgctaatactgcaggaaatgtttgttacagaagtcctagtaattcttacctgtatgacaacaatctgatcaataccaactgtgtactgactaaattttcactgctttccggatgttctccttcacctgcaccggatgtatccagctgtggattttaa

SEQ ID NO: 15 - DNA, 558 bp, synthetic construct
  misc_feature 1..558: note = DNA coding Y142D mutation of proteinglutaminase derived fromChryseobacterium proteolyticum
  source 1..558: mol_type = other DNA
ttggcgagtgtaattcctgatgtagctacattaaattctttattcaatcaaataaagaatcagtcttgcggtacctctacggcgtcctcaccatgcatcacattcagatatcctgtagacggatgttatgcaagagcccataagatgagacaaatcttaatgaacaacggctatgactgtgaaaaacaatttgtatacggaaacctaaaggcatcaacaggaacttgctgtgtggcgtggagctaccacgttgcaatattggtaagctataaaaatgcttccggagtaacggaaaaaagaattattgatccttcactattttcaagcggtcctgtaacagatacagcatggagaaacgcttgcgttaacacctcttgcggatctgcatccgtttcctcttatgctaatactgcaggaaatgttgattacagaagtcctagtaattcttacctgtatgacaacaatctgatcaataccaactgtgtactgactaaattttcactgctttccggatgttctccttcacctgcaccggatgtatccagctgtggattttaa

SEQ ID NO: 16 - DNA, 963 bp, Chryseobacterium proteolyticum
  source 1..963: mol_type = other DNA
atgaaaaatctttttttatcaatgatggcctttgtgaccgtcttaacttttaattcctgtgccgattccaacgggaatcaggaaatcaacggaaaggaaaaactaagtgtaaatgattctaagctgaaagatttcggaaagactgtaccggtagggatagacgaagaaaacggaatgataaaggtgtcatttatgttaactgcgcaattctatgaaattaagccgaccaaagaaaatgagcagtatatcggaatgcttagacaggctgttaagaatgaatctcctgtacacattttcttaaagcctaatagcaatgaaataggaaaagtggagtctgcaagtccggaagacgtaagatattttaaaacgatcctgacaaaagaagtaaaagggcaaaccaataaattggcgagtgtaattcctgatgtagctacattaaattctttattcaatcaaataaagaatcagtcttgcggtacctctacggcgtcctcaccatgcatcacattcagatatcctgtagacggatgttatgcaagagcccataagatgagacaaatcttaatgaacaacggctatgactgtgaaaaacaatttgtatacggaaacctaaaggcatcaacaggaacttgctgtgtggcgtggagctaccacgttgcaatattggtaagctataaaaatgcttccggagtaacggaaaaaagaattattgatccttcactattttcaagcggtcctgtaacagatacagcatggagaaacgcttgcgttaacacctcttgcggatctgcatccgtttcctcttatgctaatactgcaggaaatgtttattacagaagtcctagtaattcttacctgtatgacaacaatctgatcaataccaactgtgtactgactaaattttcactgctttccggatgttctccttcacctgcaccggatgtatccagctgtggattttaa

SEQ ID NO: 17 - DNA, 960 bp, Chryseobacterium sp.
  source 1..960: mol_type = other DNA
atgaaaaaatttctgttatccatgatggtattcgtgacgatgctgtcattcaatgcctgttcagattcagctgccaatcaggatcccaatcttgttgctaaagagtctaatgaaatcgccatgaaagatttcggtaaaactgttccggtagggattgaaaaagaagagggaaaatttaaagtctcttttatggtgagtgctcagccataccacattaaagacagtaaggaaaatgcaggttatatttctatgatcagacaagccgttgaaaacgaaactcctgttcatattttcctgaaaaccaacaccactgaaattgcaaaagtagataaacctactgatgatgatatccgttatttcaaatctgttttcaataaagaagagagaggagacagcaaaaaagcagtgagtgttattcctaacctggcaacactgaacagcttatttacgcagattaaaaaccaggcttgcggtacttctacagcatcttctccatgtatcactttcagatatccggtggatggatgttatgcaagagctcacaaaatgagacagatcctccttaatgcaggctacgactgtgaaaagcagttcgtttacggaaacctgagagcttctacaggaacttgctgcgtatcatgggtatatcacgtagccatattggtaagcttcaaaaatgcttccggaattgttgagaaaagaatcatcgatccttcactattctccagcggacccgtaactgacgcagcatggagagccgcttgtaccaacacaagctgtggatctgcttctgtatcttcttatgccaatacagcaggaaacgtgtactacagaagtccatcaggatctttactgtatgataacaattatgtaaataccaattgtgtattgaatatattctcatccctttcaggatgttctccttctcctgcaccaagtgtagcgagctgcggattttaa

SEQ ID NO: 18 - DNA, 960 bp, Chryseobacterium sp.
  source 1..960: mol_type = other DNA
atgaaaaaatttcttttatccatgatggtattcgtgacggtactttcatttaactcctgttcggattcaagtgccaatcaggatccgaatcttgttgctaaagagtctaatgaaattgctatgaaagactttggtaaaactgttccggtagggatagaaaaagaggatggaaagtttaaagtttcctttatagtttcagcgcagccgtatcaaattaaagatacaaaagaaaatgcgggatatatctccatgatcaaagaggctgtagaaaatgaaactcctgttcaggttttcctgaaagccaattctaacgaaatcgcaaaggtagacaaagcaacagcggatgacatccgttatttcaaatctgttttcaacaaagaagagagaggcgacagcagaaaagctgtgagcgttattcctaatcttgcaacgctgaacagcttattcactcagatcaaaaaccaggcttgcggaacttctacagcatcttcaccgtgtatcacattcagatatcctgtggatggatgctatgcgagagctcacaaaatgagacaaatccttttgaatgcaggctacgactgtgaaaaacagttcgtttacgggaacctaagagcatctacaggaacatgctgtgtgtcttgggtatatcacgtagccattttggtaagcttcaaaaatgcttccggaattgttgagaaaagaattattgatccgtcactattctccagcggacctgtaacagatactgcatggagagccgcatgtaccaacacaagctgtggatctgcttctgtttcttcttatgccaatacagcaggaaatgtatactacagaagcccatccggttctttattatatgataacaattatgtaaataccaactgtgtattgaacatattctcatccctttcaggatgttctccttcccctgcacctagtgtagcaagctgtggattttaa

SEQ ID NO: 19 - DNA, 36 bp, synthetic construct
  misc_feature 1..36: note = synthetic primer
  source 1..36: mol_type = other DNA
atctgttacaggaccgcttgaaaatagtgaaggatc

SEQ ID NO: 20 - DNA, 48 bp, synthetic construct
  misc_feature 1..48: note = synthetic primer
  source 1..48: mol_type = other DNA
acagcatggagaaacgctgttgttaacacctcttgcggatctgcatcc

SEQ ID NO: 21 - DNA, 36 bp, synthetic construct; identical to SEQ ID NO: 19
  misc_feature 1..36: note = synthetic primer
  source 1..36: mol_type = other DNA

SEQ ID NO: 22 - DNA, 48 bp, synthetic construct
  misc_feature 1..48: note = synthetic primer
  source 1..48: mol_type = other DNA
acagcatggagaaacgctgcggttaacacctcttgcggatctgcatcc

SEQ ID NO: 23 - DNA, 34 bp, synthetic construct
  misc_feature 1..34: note = synthetic primer
  source 1..34: mol_type = other DNA
ctcttgcggatctgcatccgtttcctcttatgct

SEQ ID NO: 24 - DNA, 61 bp, synthetic construct
  misc_feature 1..61: note = synthetic primer
  source 1..61: mol_type = other DNA
aatactgcaggaaatgtttgttacagaagtcctagtaattcttacctgtatgacaacaatc

SEQ ID NO: 25 - DNA, 34 bp, synthetic construct; identical to SEQ ID NO: 23
  misc_feature 1..34: note = synthetic primer
  source 1..34: mol_type = other DNA

SEQ ID NO: 26 - DNA, 61 bp, synthetic construct
  misc_feature 1..61: note = synthetic primer
  source 1..61: mol_type = other DNA
aatactgcaggaaatgttgattacagaagtcctagtaattcttacctgtatgacaacaatc